European Patent Specification EP 3 874 038 B1, published September 10, 2025. Title: Sortase F and its use in methods for conjugation. Applicant: NBE-Therapeutics. The sequence listing filed with the application follows.

SEQUENCE LISTING (93 sequences)

SEQ ID NO: 1 - protein, 183 aa, Propionibacterium acnes sortase F w/o signal peptide
TTTSSTSGIPAASAAKKGPVPAGCMKTPKPIVPVKYSIDGMKASAKVLSRGVDETGAAGAPPKNDPSSMAWFNQGPKIGSDKGNAVLTAHTYHKGGALGNRLYDKNNGIKKGDIIRLTDKTGQTVCYRYDHDTKVMVKDYNPNSNILYDNNGPAQAAIVICWDYVKKTGEFDSRVIFYTYPVA

SEQ ID NO: 2 - protein, 24 aa, Propionibacterium acnes
MVVIALIIAAIAVIFIQRNNDSDS

SEQ ID NO: 3 - protein, 40 aa, Pseudopropionibacterium propionicum
MNLVEALKNRKVQIGIAAVAVLLAVALTLVWVLQPKNDNP

SEQ ID NO: 4 - protein, 28 aa, Acidipropionibacterium acidipropionici
MIGLLVALLVIAVAATMIWRQTRDVPQA

SEQ ID NO: 5 - protein, 32 aa, Granulicoccus phenolivorans
MSKVTKSRWLPAALIAVGVIVLVVLIVVGVSA

SEQ ID NO: 6 - protein, 10 aa, Propionibacterium freudenreichii
MTRTGIRLVR

SEQ ID NO: 7 - protein, 25 aa, Propionimicrobium lymphophilum
MSGKIGKAAALLVIFLLIVAGAIYA

SEQ ID NO: 8 - protein, 43 aa, Actinobacterium LLX17
METTPQERHRHDTRRRGSAIVAVVVAIVLVALAAWWFWPEAEA

SEQ ID NO: 9 - protein, 39 aa, artificial
  WP_002530979
AGGAASSTTATTTSSTSGIPAASAAKKGPVPAGCMKTPK

SEQ ID NO: 10 - protein, 38 aa, artificial
  gi504659806
QAGATASSSGTADGAAVTSPEASSPPASPGACVTPDAA

SEQ ID NO: 11 - protein, 40 aa, artificial
  test
ATGSPASLAPASSASATPTPTPSPTPSRAAVPAGCMAKQQ

SEQ ID NO: 12 - protein, 57 aa, artificial
  test
TRTQGGTSAGEPLRVNGQTSQPEESSGGESTVAPASQDPSAASTATPGDTCTTTDQP

SEQ ID NO: 13 - protein, 73 aa, artificial
  test
LLALVALVVGLGLVAWRVVLITPSDYEKQLPTAPGAPIPDAASAGLAGTGPAHGPANGTGGGAVPAGCDPQPR

SEQ ID NO: 14 - protein, 30 aa, artificial
  test
LNNRKVDTPTPANVQTPTQPAIPEGCPTTP

SEQ ID NO: 15 - protein, 27 aa, artificial
  test
DPAPAAAPSSTAAPVETPAPCTSTATG

SEQ ID NO: 16 - protein, 27 aa, artificial
  test
PIVPVKYSIDGMKASAKVLSRGVDETG

SEQ ID NO: 17 - protein, 27 aa, artificial
  test
GFVPVRYSIESIGVEDKVISGGREEDG

SEQ ID NO: 18 - protein, 27 aa, artificial
  test
PITPSTMKIDRMKVSSPVLSLGLDTDN

SEQ ID NO: 19 - protein, 27 aa, artificial
  test
LTDPSTMYIDSMKEKSEVQSLGEEPDG

SEQ ID NO: 20 - protein, 27 aa, artificial
  test
PLVGARMTLEGHRRSMPMMSLGVAPDQ

SEQ ID NO: 21 - protein, 27 aa, artificial
  test
DIVDDPTQLLVIGTDTPLKMMSLGLDS

SEQ ID NO: 22 - protein, 27 aa, artificial
  test
PFTPTSVTVPGAIDAARVVPVPPDGEV

SEQ ID NO: 23 - protein, 53 aa, artificial
  test
AAGAPPKNDPSSMAWFNQGPKIGSDKGNAVLTAHTYHKGGALGNRLYDKNNGI

SEQ ID NO: 24 - protein, 49 aa, artificial
  test
AVAAPPKGEPRTALWWNEGPKAASNAGQVVLTIHTYQTGDAVGNMLYSD

SEQ ID NO: 25 - protein, 49 aa, artificial
  test
AAAAPPKDEPTTTAWYNRGPRPGSAKGKVVLTIHTYHKGGALGNELRQP

SEQ ID NO: 26 - protein, 50 aa, artificial
  test
TPKAPTGGEQTGWYNRSPDVGSKQGNVMMTIHTFSPKNGSNALGNRMYAP

SEQ ID NO: 27 - protein, 49 aa, artificial
  test
APASPPSHLGNTVGWFDRSVPPGAAQGRAVLTSHTFRWGGALGNELNHG

SEQ ID NO: 28 - protein, 51 aa, artificial
  test
EGAAQAPPPNEGHTVAWFTGGPKVGSPEGMATLSAHTYRYGGGLGNDLING

SEQ ID NO: 29 - protein, 49 aa, artificial
  test
SGTLPESEGRAFAWEPSPGATPGSPKGNVLMNVHTFPGDGANGNVLLDQ

SEQ ID NO: 30 - protein, 50 aa, artificial
  test
KKGDIIRLTDKTGQTVCYRYDHDTKVMVKDYNPNSNILYDNNGPAQAAIV

SEQ ID NO: 31 - protein, 55 aa, artificial
  test
NGGLLKEGAVLKLYAEDGRVACYKYTESQKIAVSEYKPESDVLERHEGDPALAIV

SEQ ID NO: 32 - protein, 54 aa, artificial
  test
GSGLTKGDLIRMTDSSGRQACYRYDHNVKVMVKDYDPDSDIIYDDHGRPMLAIV

SEQ ID NO: 33 - protein, 53 aa, artificial
  test
GALKSGDVFRITDDSGKQVCYKYSGNTKIWVASYDENSDVWHNPNGKPQLAIL

SEQ ID NO: 34 - protein, 52 aa, artificial
  test
LLAPGDVIRISDGGGRDVCYRFTGALKVRVSDYRPDSGLVYDNDGPAQLVIV

SEQ ID NO: 35 - protein, 55 aa, artificial
  test
AWTEGKTVIKISNDEGKSACYRYSGSKHLWVADYNPEVNGDLIYDDEGSPRFSLT

SEQ ID NO: 36 - protein, 52 aa, artificial
  test
LPEGGQIVLAGTAPDGSAVELCYVVSERLEMPATELLPRYYATDGPPQVAIV

SEQ ID NO: 37 - protein, 24 aa, artificial
  test
ICWDYVKKTGEFDSRVIFYTYPVA

SEQ ID NO: 38 - protein, 27 aa, artificial
  test
ICWDHNKSTNDWDSRAFIKFKPVTDAA

SEQ ID NO: 39 - protein, 25 aa, artificial
  test
ICWDYDASRNDWDSRIVFYATPVTA

SEQ ID NO: 40 - protein, 28 aa, artificial
  test
ICWDYNQPKDDWDSRIVFYADYMPMGTK

SEQ ID NO: 41 - protein, 26 aa, artificial
  test
VCSDYPLVGDAAASRALYYADLVTGP

SEQ ID NO: 42 - protein, 26 aa, artificial
  test
VCSDYPDNGSDVTLGRMIFYGDLITG

SEQ ID NO: 43 - protein, 25 aa, artificial
  test
VCSGERRGPGDWTHRTVWFASPVST

SEQ ID NO: 44 - protein, 5 aa, artificial
  test
  Xaa (3)..(3): Xaa can be any amino acid, with the exceptio of Pro
LPXTG

SEQ ID NO: 45 - protein, 5 aa, artificial
  test
  Xaa (3)..(3): Xaa can be any amino acid, with the exceptio of Pro
NPXTG

SEQ ID NO: 46 - protein, 5 aa, artificial
  test
  Xaa (3)..(3): Xaa can be any amino acid, with the exceptio of Pro
LPXTG

SEQ ID NO: 47 - protein, 5 aa, artificial
  test
  Xaa (3)..(3): Xaa can be any amino acid, with the exceptio of Pro
LPXTA

SEQ ID NO: 48 - protein, 5 aa, artificial
  test
  Xaa (3)..(3): Xaa can be any amino acid, with the exceptio of Pro
LAXTG

SEQ ID NO: 49 - protein, 5 aa, artificial
  test
LPQTG

SEQ ID NO: 50 - protein, 6 aa, artificial
  test
  Xaa (3)..(3): Xaa can be any amino acid, with the exceptio of Pro
LPXTGE

SEQ ID NO: 51 - protein, 8 aa, artificial
  test
DNPNTGDE

SEQ ID NO: 52 - protein, 9 aa, artificial
  test
  Xaa (4)..(4): Xaa can be any amino acid, with the exceptio of Pro
ENPXTNAGT

SEQ ID NO: 53 - protein, 8 aa, artificial
  test
  Xaa (4)..(4): Xaa can be any amino acid, with the exceptio of Pro
KLPXTASN

SEQ ID NO: 54 - protein, 8 aa, artificial
  test
  Xaa (4)..(4): Xaa can be any amino acid, with the exceptio of Pro
ALAXTGSE

SEQ ID NO: 55 - protein, 6 aa, artificial
  test
LPQTGE

SEQ ID NO: 56 - protein, 9 aa, artificial
  test
QALPQTGET

SEQ ID NO: 57 - protein, 6 aa, artificial
  test
LPQTGG

SEQ ID NO: 58 - protein, 31 aa, artificial
  test
AGSWSHPQFEKGGGSGGGSGGSAWSHPQFEK

SEQ ID NO: 59 - protein, 217 aa, Propionibacterium acnes sortase F
MVVIALIIAAIAVIFIQRNNDSDSAGGAASSTTATTTSSTSGIPAASAAKKGPVPAGCMKTPKPIVPVKYSIDGMKASAKVLSRGVDETGAAGAPPKNDPSSMAWFNQGPKIGSDKGNAVLTAHTYHKGGALGNRLYDKNNGIKKGDIIRLTDKTGQTVCYRYDHDTKVMVKDYNPNSNILYDNNGPAQAAIVICWDYVKKTGEFDSRVIFYTYPVA

SEQ ID NO: 60 - protein, 236 aa, Pseudopropionibacterium propionicum sortase F
MNLVEALKNRKVQIGIAAVAVLLAVALTLVWVLQPKNDNPQAGATASSSGTADGAAVTSPEASSPPASPGACVTPDAAGFVPVRYSIESIGVEDKVISGGREEDGAVAAPPKGEPRTALWWNEGPKAASNAGQVVLTIHTYQTGDAVGNMLYSDNGGLLKEGAVLKLYAEDGRVACYKYTESQKIAVSEYKPESDVLERHEGDPALAIVICWDHNKSTNDWDSRAFIKFKPVTDAA

SEQ ID NO: 61 - protein, 241 aa, Acidipropionibacterium acidipropionici sortase F
MTQNPSSENRPGHSRRTRLIGLLVALLVIAVAATMIWRQTRDVPQAATGSPASLAPASSASATPTPTPSPTPSRAAVPAGCMAKQQPITPSTMKIDRMKVSSPVLSLGLDTDNAAAAPPKDEPTTTAWYNRGPRPGSAKGKVVLTIHTYHKGGALGNELRQPGSGLTKGDLIRMTDSSGRQACYRYDHNVKVMVKDYDPDSDIIYDDHGRPMLAIVICWDYDASRNDWDSRIVFYATPVTA

SEQ ID NO: 62 - protein, 247 aa, Granulicoccus phenolivorans sortase F
MSKVTKSRWLPAALIAVGVIVLVVLIVVGVSATRTQGGTSAGEPLRVNGQTSQPEESSGGESTVAPASQDPSAASTATPGDTCTTTDQPLTDPSTMYIDSMKEKSEVQSLGEEPDGTPKAPTGGEQTGWYNRSPDVGSKQGNVMMTIHTFSPKNGSNALGNRMYAPGALKSGDVFRITDDSGKQVCYKYSGNTKIWVASYDENSDVWHNPNGKPQLAILICWDYNQPKDDWDSRIVFYADYMPMGTK

SEQ ID NO: 63 - protein, 237 aa, Propionibacterium freudenreichii sortase F
MTRTGIRLVRLLALVALVVGLGLVAWRVVLITPSDYEKQLPTAPGAPIPDAASAGLAGTGPAHGPANGTGGGAVPAGCDPQPRPLVGARMTLEGHRRSMPMMSLGVAPDQAPASPPSHLGNTVGWFDRSVPPGAAQGRAVLTSHTFRWGGALGNELNHGLLAPGDVIRISDGGGRDVCYRFTGALKVRVSDYRPDSGLVYDNDGPAQLVIVVCSDYPLVGDAAASRALYYADLVTGP

SEQ ID NO: 64 - protein, 214 aa, Propionimicrobium lymphophilum sortase F
MSGKIGKAAALLVIFLLIVAGAIYALNNRKVDTPTPANVQTPTQPAIPEGCPTTPDIVDDPTQLLVIGTDTPLKMMSLGLDSEGAAQAPPPNEGHTVAWFTGGPKVGSPEGMATLSAHTYRYGGGLGNDLINGAWTEGKTVIKISNDEGKSACYRYSGSKHLWVADYNPEVNGDLIYDDEGSPRFSLTVCSDYPDNGSDVTLGRMIFYGDLITG

SEQ ID NO: 65 - protein, 223 aa, actinobacterium LLX17 sortase F
METTPQERHRHDTRRRGSAIVAVVVAIVLVALAAWWFWPEAEADPAPAAAPSSTAAPVETPAPCTSTATGPFTPTSVTVPGAIDAARVVPVPPDGEVSGTLPESEGRAFAWEPSPGATPGSPKGNVLMNVHTFPGDGANGNVLLDQLPEGGQIVLAGTAPDGSAVELCYVVSERLEMPATELLPRYYATDGPPQVAIVVCSGERRGPGDWTHRTVWFASPVST

SEQ ID NO: 66 - protein, 229 aa, Actinomadura atramentaria sortase F
MARRCPWGRAAARRTGRNRCAPPAPQPPPGCRFGRDAAPVPFPHETPYADHAPDAPGADRLRPIPLTGDLGDALPCTIAIPAIGVSAALAGVGRDAAGRVAAPPADEPGLAGWYAAGPTPGRPGAAVIVGNPLGSPGAGFARLGDLACGDIVGIVRADDTVAVFRVTGTERVPWDDFPESRVHGPVDGPELRLIAGAGRYDADARSHPARVIVYAAFTAAYRLTDLASL

SEQ ID NO: 67 - protein, 309 aa, Granulicoccus phenolivorans sortase F
MLLLLSPLAIFGAIFWPARSSEQVSAAPAWPADPASPAAPSTDGDGAPEPAATMPTLQVPEPDPVPANEPPATPQPAAEAGPGTGDSGQPGADRQGAGQQGAGQQGAGQQGAGQQGAGQQEAGKSGTTGSGTTGSGTTGSGQSANEGGRCVSSGGSFTGVTRFQLSRMGVDVPLRPVGEDSTGAPGAPPLNQMYSAAWYNKSPRPGSGQGNVIINIHSWASGAALGNDLRTGIRSGDVIRVVGDGGQVACYRFRDMIKFRVADYDPRSGIYHNKSGRPQLAIMTCWDRNKSTGEYESRVIMYADYVARA

SEQ ID NO: 68 - protein, 250 aa, Propionibacteriaceae bacterium P6A17 sortase F
MQQLRRRRIVATIVALVVLVAGGLLLRQGLSRTALLEQPETSVALPSRETPPPTSAPPTTAPPSPWPSPTPSPTPTASPSPSAATAQCSHSTSGFTPTSFTLARVGAKERVIAMRTQGGQISAPPKNDRRSAGWWSDGPRPGADHGKVVLTIHTYRPSLRPALGNELYDGGESALRPGDVPQLHAKDGCTVCYEFVEAQRIMVADYDPSSRVMLDPDGEPSAVIVICWDFSSSTKDWDSRVFFQFRRVTG

SEQ ID NO: 69 - protein, 236 aa, Pseudopropionibacterium propionicum sortase F; identical to SEQ ID NO: 60

SEQ ID NO: 70 - protein, 269 aa, Aestuariimicrobium kwangyangense sortase F
MADQAPVPASPQPDGVPGRGRSSSPGRGPSRLVVLLVVLVILVGAGFAIWRATNRQPGVAAPPASPETSTSATIVAPTPESPTSSGTTPAQPTPTASSSTPLPPGCSSPTAPMDDPQRLSIESMKVDSPMLSLGLDESGSAAAPPKDQPRTVGWFDQGPKLGSGQGHAVLTIHTYRNGNALGNELADPNSGLRPGALVRVSDGRGNTVCYTFSRSTKVWVKDYDPNSTVLYDDAGAPEAIIVICWDFNRATAAWDSRILFHLTPVAPSA

SEQ ID NO: 71 - protein, 241 aa, Acidipropionibacterium acidipropionici sortase F; identical to SEQ ID NO: 61

SEQ ID NO: 72 - protein, 258 aa, Cutibacterium acnes KPA171202 sortase F
MTDRSPRRQEPSTGSTPSNSSTTHAGDSAQPGGPKWRIVALVVVIALIIAAIAVIFIQRNNDSDSAGGAASSTTATTTSSTSGIPAASAAKKGPVPAGCMKTPKPIVPVKYSIDGMKASAKVLSRGVDETGAAGAPPKNDPSSMAWFNQGPKIGSDKGNAVLTAHTYHKGGALGNRLYDKNNGIKKGDIIRLTDKTGQTVCYRYDHDTKVMVKDYNPNSNILYDNNGPAQAAIVICWDYVKKTGEFDSRVIFYTYPVA

SEQ ID NO: 73 - protein, 187 aa, Rhodococcus sp. AD45 sortase F
MLFLLLPGCAVSGQARLEAAHTSVDTIPADSLQSQSVPMAQPTRLSIADLGIDATVLPMPAGACPVLDPPTLADAYWVGCRSEPGTDSDGTVFVIGHAGAGTAAVFDTLPDIVAGSRVLIETDSGTLEYTVRSTALYEKFGEAQESPELRLRQPGRLVLVTCYLENGTTLSSKNFVAYAEITGALAR

SEQ ID NO: 74 - protein, 187 aa, Rhodococcus sp. AD45 sortase F; identical to SEQ ID NO: 73

SEQ ID NO: 75 - protein, 241 aa, Corynebacterium otitidis sortase F
MTHDADAQHSQPDGGDQAADEDHKRRSPVGIIIAVVAVVALVIGIGAWAISSNSGDDEENPIAGQEAAPEEDIPPVDDSGEQEHELEPAPGEREGVEGMAISVDGETAPVDFVQVTDQGVLLPPQDVSRVGWYSASAIPGEYGEGSSVITGHVNFAGQGEGFARRFVDLAEGSEVIVHVNGEDRAFRVSEPPEHVTKGDALPEVVNQAEGDNRLVLITCGGEFVGGQLGYADNVITVADPV

SEQ ID NO: 76 - protein, 221 aa, Corynebacterium camporealensis sortase F
MEAKESSIDEHSHKAGASRWILLLLTVVLIALLAGVALYAGLRSSETSDSGAGEQLPVAQTDLPEPAPGIRDGVNEMQLKIGGESAKVEFVQLTDQGALIPPEDVSKVGWYSASAVPGQEGPTVGTSVITGHVNEIDQGDGFAAKFPELRPGDVVSVIVDGEERQFTVSKDPIRVVKGAELPESVNRSTGENELVLITCGGEFVGGTLGYADNIVVEATPL

SEQ ID NO: 77 - protein, 249 aa, Actinobacteria sortase F
MAAEQHGGGAPSVPADDRGGRRPGRRTGLLLAAGAITVAAGIAIAVTAPSPGPAAAGDGAGSGRQAPPPVTVAPAPVPGPGEPEPVAPAPVPARADTGDAPNRLILPDGSAASVDTIAPTGRGALHPPTDPGRVGWWVDSALPGSGTGAVVVTGHINWAGHAGFARRWLPPSAGGRVEPGQDITLSTTGSGPRRYRVTGTRAYDKRSGLPSEVNRRTGPETLLLITCGGRWAGGDLGYADNLITTAQPA

SEQ ID NO: 78 - protein, 206 aa, Rhodococcus sp. AD45 sortase F
MTQSSRQTLRRLCGAAALTVLLCVSGCSDDSDQPVRVLATGQEDLPSALEAVVDNPATPTQLRIGSEAAVVLAIKTTSGGSLIPPEDVSKVGWWADSAFPGSGTGTVVITGHINDVYAGDGFGKKFSALTPGSVVTLTGEDGHEWTYRIDAVDEYRKDGELPVERLNRMDGPETLALITCGGEFVGPPLGYEDNDIAWATRIPDLS

SEQ ID NO: 79 - protein, 202 aa, Gordonia phthalatica sortase F
MRRLIRILCTLAAVAALVATAACGTEEATPSTSSTQAQENLRPPVSAVSHDPSTPKSVVIDGASAPTVSVATDAAGTLLPPTDIAKLGWWVDSALPGSGAGTIVVAGHVDDLKQGTGYAARFAKLTAGDTVTVDTADGAKHTYRVTRVVDAQKEGKGADAVPFDELNRLDGPETLALVTCGGPFIGPPLGYRDNIVVFATPA

SEQ ID NO: 80 - protein, 182 aa, Gordonia jacobaea sortase F
MTLLVGCSTRTSESSVATPSAQTQLPAPVAARTDEPAAPKSIEVGGDSAVTDAVATDTTGALLPPQDVHRLGWWVDSALPGSGKGTIVVTGHVDEASQGRGFAARFSSLAPGTEVAVTTAKGETVHYRVRNVQKADKEKGFPAAELNRLDGPETLALVTCGGAFVGPPLGYADNIIAWATRA

SEQ ID NO: 81 - protein, 194 aa, Tsukamurella paurometabola sortase F
MRRLSGLVLAVAVLAAGCGTVEGTAEPVPSNPAAQSDLRAPVVATANESAAPVRVSASGSDAPVDGVATDAQGALYPPQDVGRVGWWIDSALPGSGRGSVVVTGHIDDARQGDGFAKRFGALRAGDTVSLTGKDGRTIAYRVTRTMSVGKGALPVGDLNRQDGPETLILVTCGGRFVGPPMGYENNDLVYAERA

SEQ ID NO: 82 - protein, 199 aa, Gordonia otitidis sortase F
MNGPRMRALFCLVALGFALVIGGCSTSDRESAATAPSAQAELPAPVAARTDEKSAPKSIAVGGDSAITEAVATDTTGALLPPQDVRRLGWWVDSSLPGSGKGTIVVTGHVNEADQGTGFAARFATMKPGETVAVTTASGQQINYRVTRIQNADKETGFPSDELNRVDGPETLALVTCGGQFVGPPLGYKDNVIAWATRA

SEQ ID NO: 83 - protein, 251 aa, Corynebacterium sortase F
MTDQFGSDETGKEPGNTPGIEPETETGALDHVDPFDQAEDPADSQVEDLQDVPWWKQPRVYIAAIALIGVIALLVIAQLHRNDSALEGAQENLPTPAQGSRGAVHEMEMLIDGKSAPIDFVQLTDQGSLIPPTDVSRLGWYSASAIPGEKGAAGSSVITGHVNEVDQGDGYAARFADLKAGDTVTVKVDGESRDFTVSKDPIQVVKGAQMPEAVNDAVGENRLVLITCGGEFVGGTLGYADNIIVEATPVR

SEQ ID NO: 84 - protein, 289 aa, Streptococcus suis sortase F
MIKWLKKKGPSFIMPLIFILGIGLLAYPSVSDYWNSFHQSEAIMSYSDTVSDMTADQYKEIIDSARQYNQEKPLNWNVTASDIEAYNQELNFNKDGIMGYIEIPKIDVKLSIFHGTDETVLETSIGHLEGTSLPVGGLGTHSVLSGHRGLPSARLFSDLDKLREGDIFTIHVLNETLTYKVDQIRVVEPSDLSALTMEPQKDLLTLVTCTPYGINTHRLLVRGYRIENVNGSALVTSDAIQIKAIFIAPFIATPILFVILIYIFITTSKTFRSRNRNQVLDDFLVPKKF

SEQ ID NO: 85 - protein, 200 aa, Gordonia neofelifaecis sortase F
MKIYQAAVTSVAAAALVFTAACAADGGDSPPPGTAQANLPAPVRAASDAPSTPVDLTIDGAAAAIDAVATDTAGALLPPRDVHRLGWWVDSSLPGSGSGAIVVTGHVDDVQQGSGFASRFTTLRTGDTVDLTTTDGHRHDYRITRTVLADKEATGSGGLPVAELNRRDGPETLALITCGGPFIGPPLGYRDNVVVFAVPV

SEQ ID NO: 86 - protein, 117 aa, antibody sequence
QIQLQQSGPEVVKPGASVKISCKASGYTFTDYYITWVKQKPGQGLEWIGWIYPGSGNTKYNEKFKGKATLTVDTSSSTAFMQLSSLTSEDTAVYFCANYGNYWFAYWGQGTQVTVSA

SEQ ID NO: 87 - protein, 111 aa, antibody sequence
DIVLTQSPASLAVSLGQRATISCKASQSVDFDGDSYMNWYQQKPGQPPKVLIYAASNLESGIPARFSGSGSGTDFTLNIHPVEEEDAATYYCQQSNEDPWTFGGGTKLEIK

SEQ ID NO: 88 - protein, 5 aa, antibody sequence
DYYIT

SEQ ID NO: 89 - protein, 17 aa, antibody sequence
WIYPGSGNTKYNEKFKG

SEQ ID NO: 90 - protein, 8 aa, antibody sequence
YGNYWFAY

SEQ ID NO: 91 - protein, 15 aa, antibody sequence
KASQSVDFDGDSYMN

SEQ ID NO: 92 - protein, 7 aa, antibody sequence
AASNLES

SEQ ID NO: 93 - protein, 9 aa, antibody sequence
QQSNEDPWT